European Patent Specification EP 3 423 838 B1, published November 8, 2023. Title: METHODS AND COMPOSITIONS FOR THE DETECTION AND DIAGNOSIS OF RENAL DISEASE AND PERIODONTAL DISEASE. Applicant: Yerramilli, Mahalakshmi Farace, Giosi Quinn, John J Yerramilli, Murthy V.S.N. The sequence listing filed with the application follows.

SEQUENCE LISTING (27 sequences)

SEQ ID NO: 1 - protein, 77 aa, Canis familiaris
QVKAQLEERENKKYTTFKAVTFRSQVVAGTPYFIKVQVDDDEFVHLRVFQSLPHENKPLALSSYQTNKAKHDELAYF

SEQ ID NO: 2 - protein, 21 aa, Canis familiaris
MMCGAPSASQPATADTQAIAD

SEQ ID NO: 3 - protein, 98 aa, Canis familiaris
  MISC_FEATURE (52)..(52): The X stands for any amino acid
MMCGAPSASQPATADTQAIADQVKAQLEERENKKYTTFKAVTFRSQVVAGTXYFIKVQVDDDEFVHLRVFQSLPHENKPLALSSYQTNKAKHDELAYF

SEQ ID NO: 4 - protein, 13 aa, Canis familiaris
QTNKAKHDELAYF

SEQ ID NO: 5 - protein, 18 aa, Canis familiaris
CGAPSASQPATADTQAIA

SEQ ID NO: 6 - protein, 8 aa, Canis familiaris
CGAPSASQ

SEQ ID NO: 7 - protein, 9 aa, Canis familiaris
CAIADQVKA

SEQ ID NO: 8 - protein, 15 aa, Canis familiaris
FQSLPHENKPLALSS

SEQ ID NO: 9 - protein, 18 aa, Canis familiaris
SQVVAGTPYFIKVQVDDD

SEQ ID NO: 10 - protein, 8 aa, Canis familiaris
KHDELAYF

SEQ ID NO: 11 - protein, 29 aa, Canis familiaris
MMCGAPSASQPATADTQAIADQVKAQLEE

SEQ ID NO: 12 - protein, 8 aa, Canis familiaris
AIADQVKA

SEQ ID NO: 13 - protein, 18 aa, Canis familiaris
SQVVAGTNYFIKVQVDDD

SEQ ID NO: 14 - protein, 98 aa, Homo sapiens
MMCGAPSATQPATAETQHIADQVRSQLEEKENKKFPVFKAVSFKSQVVAGTNYFIKVHVGDEDFVHLRVFQSLPHENKPLTLSNYQTNKAKHDELTYF

SEQ ID NO: 15 - protein, 13 aa, Homo sapiens
QTNKAKHDELTYF

SEQ ID NO: 16 - protein, 12 aa, Canis familiaris
QTNKAKHDELAY

SEQ ID NO: 17 - protein, 11 aa, Canis familiaris
QTNKAKHDELA

SEQ ID NO: 18 - protein, 10 aa, Canis familiaris
QTNKAKHDEL

SEQ ID NO: 19 - protein, 9 aa, Canis familiaris
QTNKAKHDE

SEQ ID NO: 20 - protein, 4 aa, Canis familiaris
LAYF

SEQ ID NO: 21 - protein, 5 aa, Canis familiaris
ELAYF

SEQ ID NO: 22 - protein, 6 aa, Canis familiaris
DELAYF

SEQ ID NO: 23 - protein, 7 aa, Canis familiaris
HDELAYF

SEQ ID NO: 24 - protein, 9 aa, Canis familiaris
AKHDELAYF

SEQ ID NO: 25 - protein, 10 aa, Canis familiaris
KAKHDELAYF

SEQ ID NO: 26 - protein, 11 aa, Canis familiaris
NKAKHDELAYF

SEQ ID NO: 27 - protein, 12 aa, Canis familiaris
TNKAKHDELAYF